European Patent Specification EP 3 733 866 B1, published November 15, 2023. Title: OPTICAL ANALYTE DETECTION SYSTEMS AND METHODS OF USE. Applicant: Genalyte, Inc. Bailey, Ryan C. Qavi, Abraham J. Kindt, Jared T. Byeon, Ji-Yeon Luchansky, Matthew S. McClellan, Melinda S. Washburn, Adam L. Owen, Tate Gleeson, Martin Anthony Gunn, III, Lawrence C. The sequence listing filed with the application follows.

SEQUENCE LISTING (14 sequences)

SEQ ID NO: 1 - RNA, 22 nt, Homo sapiens
uagcagcacguaaauauuggcg

SEQ ID NO: 2 - RNA, 22 nt, Homo sapiens
uagcuuaucagacugauguuga

SEQ ID NO: 3 - RNA, 22 nt, Homo sapiens
uggcucaguucagcaggaacag

SEQ ID NO: 4 - RNA, 22 nt, Homo sapiens
uucaaguaauccaggauaggcu

SEQ ID NO: 5 - DNA, 22 bp, Artificial Sequence
  Synthetic oligo
atcgtcgtgcatttataaccgc

SEQ ID NO: 6 - DNA, 22 bp, Artificial Sequence
  Synthetic oligo
atcgaatagtctgactacaact

SEQ ID NO: 7 - DNA, 22 bp, Artificial Sequence
  Synthetic oligo
ctgttcctgctgaactgagcca

SEQ ID NO: 8 - DNA, 22 bp, Artificial Sequence
  Synthetic oligo
aagttcattaggtcctatccga

SEQ ID NO: 9 - RNA, 10 nt, Artificial Sequence
  Synthetic oligo
aaaggugcgu

SEQ ID NO: 10 - RNA, 20 nt, Artificial Sequence
  Synthetic oligo
aaaggugcguuuauagaucu

SEQ ID NO: 11 - RNA, 40 nt, Artificial Sequence
  Synthetic oligo
aaaggugcguuuauagaucuagacuagguugcagcaacua

SEQ ID NO: 12 - DNA, 40 bp, Artificial Sequence
  Synthetic oligo
tagttgctgcaacctagtctagatctataaacgcaccttt

SEQ ID NO: 13 - DNA, 54 bp, Artificial Sequence
  Synthetic oligo
ctgttcctgctgaactgagccaaaaaaaaaaactgttcctgctgaactgagcca

SEQ ID NO: 14 - DNA, 22 bp, Artificial Sequence
  Synthetic oligo
ctgttcctgctgaactgagcca